European Patent Application EP 4 574 165 A1, published June 25, 2025. Title: IMMUNOCYTOKINE FOR CANCER TREATMENT. Applicant: EGLE THERAPEUTICS. The sequence listing filed with the application follows.

SEQUENCE LISTING (17 sequences)

SEQ ID NO: 1 - protein, 133 aa, Homo sapiens [sequence omitted]

SEQ ID NO: 2 - protein, 10 aa, synthetic construct
GFTFSSYTMH

SEQ ID NO: 3 - protein, 17 aa, synthetic construct
FISYDGNNKYYADSVKG

SEQ ID NO: 4 - protein, 11 aa, synthetic construct
ARTGWLGPFDY

SEQ ID NO: 5 - protein, 12 aa, synthetic construct
RASQSVGSSYLA

SEQ ID NO: 6 - protein, 7 aa, synthetic construct
GAFSRAT

SEQ ID NO: 7 - protein, 9 aa, synthetic construct
QQYGSSPWT

SEQ ID NO: 8 - protein, 118 aa, synthetic construct
QVQLVESGGGVVQPGRSLRLSCAASGFTFSSYTMHWVRQAPGKGLEWVTFISYDGNNKYYADSVKGRFTISRDNSKNTLYLQMNSLRAEDTAIYYCARTGWLGPFDYWGQGTLVTVSS

SEQ ID NO: 9 - protein, 108 aa, synthetic construct
EIVLTQSPGTLSLSPGERATLSCRASQSVGSSYLAWYQQKPGQAPRLLIYGAFSRATGIPDRFSGSGSGTDFTLTISRLEPEDFAVYYCQQYGSSPWTFGQGTKVEIK

SEQ ID NO: 10 - protein, 16 aa, synthetic construct
GGGGGSGGGGSGGGGS

SEQ ID NO: 11 - protein, 594 aa, synthetic construct
QVQLVESGGGVVQPGRSLRLSCAASGFTFSSYTMHWVRQAPGKGLEWVTFISYDGNNKYYADSVKGRFTISRDNSKNTLYLQMNSLRAEDTAIYYCARTGWLGPFDYWGQGTLVTVSSASTKGPSVFPLAPSSKSTSGGTAALGCLVKDYFPEPVTVSWNSGALTSGVHTFPAVLQSSGLYSLSSVVTVPSSSLGTQTYICNVNHKPSNTKVDKRVEPKSCDKTHTCPPCPAPELLGGPSVFLFPPKPKDTLMISRTPEVTCVVVDVSHEDPEVKFNWYVDGVEVHNAKTKPREEQYNSTYRVVSVLTVLHQDWLNGKEYKCKVSNKALPAPIEKTISKAKGQPREPQVYTLPPSRDELTKNQVSLTCLVKGFYPSDIAVEWESNGQPENNYKTTPPVLDSDGSFFLYSKLTVDKSRWQQGNVFSCSVMHEALHNHYTQKSLSLSPGGGGGSGGGGSGGGGSAPTSSTKETQEQLERLLRDLQLILKGINNPKNPKLTRMLTFKFYMPKKATELKHLQCLEEELKPLEEVLNLAQSKNFHLRPRDLINNINKIVLKLKGSETTFMCEYADETATIVEFLKRWIAFCQKIISTLT

SEQ ID NO: 12 - protein, 215 aa, synthetic construct
EIVLTQSPGTLSLSPGERATLSCRASQSVGSSYLAWYQQKPGQAPRLLIYGAFSRATGIPDRFSGSGSGTDFTLTISRLEPEDFAVYYCQQYGSSPWTFGQGTKVEIKRTVAAPSVFIFPPSDEQLKSGTASVVCLLNNFYPREAKVQWKVDNALQSGNSQESVTEQDSKDSTYSLSSTLTLSKADYEKHKVYACEVTHQGLSSPVTKSFNRGEC

SEQ ID NO: 13 - protein, 132 aa, synthetic construct
APTSSTKETQEQLERLLRDLQLILKGINNYKNPKLTRMLTFKFYMPKKATELKHLQCLEEELKPLEEVLNLAQSKNFHLRPRDLINNINKIVLKLKGSETTFMCEYADETATIVEFLKRWIAFCQKIISTLT

SEQ ID NO: 14 - protein, 132 aa, synthetic construct
APTSSTKETQEQLERLLRDLQLILKGINNPKNPKLTRMLTFKFYMPKKATELKHLQCLEEELKPLEEVLNLAQSKNFHLRPRDLINNINKIVLKLKGSETTFMCEYADETATIVEFLKRWIAFCQKIISTLT

SEQ ID NO: 15 - protein, 132 aa, synthetic construct
APTSSTKETQEQLERLLRDLQLILKGINNYKNPKLTRMLTFKFYMPKQATSLKHLQCLEEELKPLEEVLNLAQSKNFHLEPRNLINNINKIVLKLKGSETTFMCEYADETATIVEFLKRWIAFCQSIISRST

SEQ ID NO: 16 - DNA, 1839 bp, synthetic construct
  source 1..1839: mol_type = other DNA
atggagttcggactgtcctgggtattcctcgtggcgatcatcaagggcgtccagtgccaagtgcagctggtggagtccggtggcggagtcgtacagcccggtcggtcgctgcgcctctcgtgcgcagcgagcgggttcaccttctcgtcctacaccatgcactgggtacgtcaggcaccgggcaagggcctggagtgggtcacgttcatcagctatgacggcaacaacaagtactacgccgactcggtcaagggcaggttcaccatctcgcgtgacaactccaagaacaccctctacctccagatgaactccctccgcgcagaggacaccgcgatctactactgcgcgcgaaccggttggctgggcccgttcgactactggggccagggcacgctcgtgaccgtttcgagcgcctccaccaagggcccgagcgtcttccccctggcgccaagcagcaagagcaccagcggaggaacggctgccctgggctgcctggtgaaggactacttcccggagccggtcacggtatcgtggaacagtggcgcgctgacgtccggcgtccacaccttccccgcggtgctccagtcgagcggcctgtactcgctgtcgtcggtagtcacggtcccctcgtcctcgctcggcacgcagacctacatctgcaacgtgaatcacaagccgtccaacacgaaggtggacaagcgcgtcgagcccaagtcctgcgacaagacgcacacttgcccgccctgccctgccccggagctccttggcggtccgtccgtcttcctgttccccccgaagccgaaggacaccctgatgatctcccgcaccccggaggtgacctgcgtcgtggtggacgtgtcccacgaggaccctgaggtgaaattcaactggtacgtggacggcgtcgaagtccacaacgccaagaccaagccgcgtgaggagcagtacaattccacctaccgcgtggtgtccgtgctgacggtgctgcaccaggactggctgaacggcaaggagtacaagtgcaaggtgtccaacaaagccctcccggctcccatcgagaagaccatctccaaggccaagggccagccccgtgaaccccaggtctacaccctccccccctcgcgcgatgagctgacgaagaaccaggtgagcctgacctgcctcgtcaagggcttctatccgtccgacatcgcggtcgagtgggaatcgaacggccagcccgagaacaattacaagaccaccccgccagtgctcgactccgatggcagcttcttcctttactcgaagctcacggtcgacaagagccgttggcagcagggcaacgtgttcagctgctcggtcatgcacgaggccttgcacaaccactacacgcaaaagagcctctccctgagcccgggtggtgggggtggctcgggcgggggcggcagcggcggaggcggctcggcacccaccagtagcaccaaggaaacccaggagcaactggagaggctgctgagggacctgcagctgatcctgaaggggatcaacaaccctaagaacccgaagctgacccgcatgctgaccttcaagttctacatgccgaagaaggcgaccgaattgaagcacctgcagtgcctggaggaagagctgaagcccctggaggaggtcctcaacctcgcacagtccaagaacttccacctccgtccgcgggacctcatcaacaacatcaacaagatcgtcctcaagctcaaaggctcggaaaccaccttcatgtgcgagtacgccgacgaaacggccaccatcgtcgagttcctgaagcgctggatcgccttctgccagaagatcatctccacgctgacc

SEQ ID NO: 17 - DNA, 711 bp, synthetic construct
  source 1..711: mol_type = other DNA
atggacatgcgcgtgcctgcgcagctcctgggcctcctcctgctgtggctcaggggggcacgctgcgagatcgtcttgacgcagagtccggggaccctcagcctgagccccggagagcgggctaccctgagctgtcgtgcgtcgcagagcgtcggctcgtcctacttggcgtggtaccagcagaagccgggacaggcaccgcgcctcctgatctacggcgccttcagccgcgcaacgggcatccccgaccgcttctccggatcgggcagcggcaccgacttcactctgacgatctcacggctggagcccgaggacttcgccgtctactactgccagcagtacggcagcagcccgtggaccttcggccagggcaccaaggtggagatcaagcggaccgtggccgcaccgtcggtcttcatcttccccccgagcgacgagcagctgaagtcaggtaccgccagcgtggtctgcctgctgaataacttctaccccagggaggcgaaggtgcagtggaaggtcgacaacgccctccagtccggtaactcccaggagagcgtcaccgagcaggactccaaggactccacctactccctctcctcgacgctcaccctgtccaaggccgactacgaaaagcacaaggtctacgcgtgcgaggtgacgcaccagggcctgtcttcgccggtcacgaagtcgttcaaccggggtgagtgc